European Patent Specification EP 3 728 165 B1, published June 18, 2025. Title: Stimulation de la nitrification d'un sol avec des compositions comprenant un extrait de plante. Applicant: Agro Innovation International. The sequence listing filed with the application follows.

SEQUENCE LISTING (4 sequences)

SEQ ID NO: 1 - DNA, 19 bp, Artificial Sequence
  AOA-amoA F
saatggtctggcttagacg

SEQ ID NO: 2 - DNA, 20 bp, Artificial Sequence
  AOA-amoA R
gcggccatccatctgtatgt

SEQ ID NO: 3 - DNA, 18 bp, Artificial Sequence
  AOB-amoA F
ggggtttctactggtggt

SEQ ID NO: 4 - DNA, 22 bp, Artificial Sequence
  AOB-amoA R
ccccttcgggaaagccttcttc